European Patent Application EP 4 306 955 A2, published January 17, 2024. Title: INTEGRATED FUNCTIONAL AND MOLECULAR PROFILING OF CELLS. Applicant: University of Houston System. Application EP. The sequence listing filed with the application follows.

SEQUENCE LISTING (190 sequences)

SEQ ID NO: 1 - DNA, 17 bp, synthetic construct
  misc_feature 1..17: note = Primer for DELTAgene qPCR assay in Example 2
  source 1..17: mol_type = other DNA
ccatggcgaccgtcaca

SEQ ID NO: 2 - DNA, 19 bp, synthetic construct
  misc_feature 1..19: note = Primer for DELTAgene qPCR assay in Example 2
  source 1..19: mol_type = other DNA
tcactctggcctccagaca

SEQ ID NO: 3 - DNA, 18 bp, synthetic construct
  misc_feature 1..18: note = Primer for DELTAgene qPCR assay in Example 2
  source 1..18: mol_type = other DNA
tccgtggccttagctgtg

SEQ ID NO: 4 - DNA, 22 bp, synthetic construct
  misc_feature 1..22: note = Primer for DELTAgene qPCR assay in Example 2
  source 1..22: mol_type = other DNA
cccagacacatagcaattcagg

SEQ ID NO: 5 - DNA, 22 bp, synthetic construct
  misc_feature 1..22: note = Primer for DELTAgene qPCR assay in Example 2
  source 1..22: mol_type = other DNA
gacagaggatcatgctgtactt

SEQ ID NO: 6 - DNA, 19 bp, synthetic construct
  misc_feature 1..19: note = Primer for DELTAgene qPCR assay in Example 2
  source 1..19: mol_type = other DNA
cttggcatgagatgcagga

SEQ ID NO: 7 - DNA, 19 bp, synthetic construct
  misc_feature 1..19: note = Primer for DELTAgene qPCR assay in Example 2
  source 1..19: mol_type = other DNA
aacccctcagagcacacaa

SEQ ID NO: 8 - DNA, 20 bp, synthetic construct
  misc_feature 1..20: note = Primer for DELTAgene qPCR assay in Example 2
  source 1..20: mol_type = other DNA
cggccccggaaaattgaata

SEQ ID NO: 9 - DNA, 23 bp, synthetic construct
  misc_feature 1..23: note = Primer for DELTAgene qPCR assay in Example 2
  source 1..23: mol_type = other DNA
tcccatatctggacatctggaac

SEQ ID NO: 10 - DNA, 23 bp, synthetic construct
  misc_feature 1..23: note = Primer for DELTAgene qPCR assay in Example 2
  source 1..23: mol_type = other DNA
ctcctgctaagatggagtgttca

SEQ ID NO: 11 - DNA, 20 bp, synthetic construct
  misc_feature 1..20: note = Primer for DELTAgene qPCR assay in Example 2
  source 1..20: mol_type = other DNA
ccgtcacctgctcagaatca

SEQ ID NO: 12 - DNA, 19 bp, synthetic construct
  misc_feature 1..19: note = Primer for DELTAgene qPCR assay in Example 2
  source 1..19: mol_type = other DNA
ccatggtgcagaggaggac

SEQ ID NO: 13 - DNA, 20 bp, synthetic construct
  misc_feature 1..20: note = Primer for DELTAgene qPCR assay in Example 2
  source 1..20: mol_type = other DNA
cgtgactgtcctgtctctcc

SEQ ID NO: 14 - DNA, 22 bp, synthetic construct
  misc_feature 1..22: note = Primer for DELTAgene qPCR assay in Example 2
  source 1..22: mol_type = other DNA
tctaccacaaagttgcgaggaa

SEQ ID NO: 15 - DNA, 20 bp, synthetic construct
  misc_feature 1..20: note = Primer for DELTAgene qPCR assay in Example 2
  source 1..20: mol_type = other DNA
aacccagaaagccccagaaa

SEQ ID NO: 16 - DNA, 22 bp, synthetic construct
  misc_feature 1..22: note = Primer for DELTAgene qPCR assay in Example 2
  source 1..22: mol_type = other DNA
gtggtgtttggagtttccatcc

SEQ ID NO: 17 - DNA, 20 bp, synthetic construct
  misc_feature 1..20: note = Primer for DELTAgene qPCR assay in Example 2
  source 1..20: mol_type = other DNA
acataccaggactgcctgag

SEQ ID NO: 18 - DNA, 21 bp, synthetic construct
  misc_feature 1..21: note = Primer for DELTAgene qPCR assay in Example 2
  source 1..21: mol_type = other DNA
gtggatgtactggggaaatgc

SEQ ID NO: 19 - DNA, 20 bp, synthetic construct
  misc_feature 1..20: note = Primer for DELTAgene qPCR assay in Example 2
  source 1..20: mol_type = other DNA
cattgcctcacagaccttcc

SEQ ID NO: 20 - DNA, 21 bp, synthetic construct
  misc_feature 1..21: note = Primer for DELTAgene qPCR assay in Example 2
  source 1..21: mol_type = other DNA
agggtggtgtctgctatatcc

SEQ ID NO: 21 - DNA, 21 bp, synthetic construct
  misc_feature 1..21: note = Primer for DELTAgene qPCR assay in Example 2
  source 1..21: mol_type = other DNA
tgagacatccgttcccctaca

SEQ ID NO: 22 - DNA, 20 bp, synthetic construct
  misc_feature 1..20: note = Primer for DELTAgene qPCR assay in Example 2
  source 1..20: mol_type = other DNA
tggcagggctccgatgtata

SEQ ID NO: 23 - DNA, 19 bp, synthetic construct
  misc_feature 1..19: note = Primer for DELTAgene qPCR assay in Example 2
  source 1..19: mol_type = other DNA
aggcagcgatgtctgtgaa

SEQ ID NO: 24 - DNA, 19 bp, synthetic construct
  misc_feature 1..19: note = Primer for DELTAgene qPCR assay in Example 2
  source 1..19: mol_type = other DNA
agctcaagccccaacatca

SEQ ID NO: 25 - DNA, 19 bp, synthetic construct
  misc_feature 1..19: note = Primer for DELTAgene qPCR assay in Example 2
  source 1..19: mol_type = other DNA
gtggtggctctccttgtca

SEQ ID NO: 26 - DNA, 21 bp, synthetic construct
  misc_feature 1..21: note = Primer for DELTAgene qPCR assay in Example 2
  source 1..21: mol_type = other DNA
tgtggtgttgtctccgatgta

SEQ ID NO: 27 - DNA, 22 bp, synthetic construct
  misc_feature 1..22: note = Primer for DELTAgene qPCR assay in Example 2
  source 1..22: mol_type = other DNA
agaagccagaagtcaggtatcc

SEQ ID NO: 28 - DNA, 20 bp, synthetic construct
  misc_feature 1..20: note = Primer for DELTAgene qPCR assay in Example 2
  source 1..20: mol_type = other DNA
tcccgtcactgtgtagttcc

SEQ ID NO: 29 - DNA, 22 bp, synthetic construct
  misc_feature 1..22: note = Primer for DELTAgene qPCR assay in Example 2
  source 1..22: mol_type = other DNA
agaagggaaggagtacacagac

SEQ ID NO: 30 - DNA, 20 bp, synthetic construct
  misc_feature 1..20: note = Primer for DELTAgene qPCR assay in Example 2
  source 1..20: mol_type = other DNA
ccgggtgcagtttatttcca

SEQ ID NO: 31 - DNA, 19 bp, synthetic construct
  misc_feature 1..19: note = Primer for DELTAgene qPCR assay in Example 2
  source 1..19: mol_type = other DNA
agtgcacagcagggaacaa

SEQ ID NO: 32 - DNA, 19 bp, synthetic construct
  misc_feature 1..19: note = Primer for DELTAgene qPCR assay in Example 2
  source 1..19: mol_type = other DNA
aggctgcctcctccacata

SEQ ID NO: 33 - DNA, 20 bp, synthetic construct
  misc_feature 1..20: note = Primer for DELTAgene qPCR assay in Example 2
  source 1..20: mol_type = other DNA
aaccacagcccttccttcaa

SEQ ID NO: 34 - DNA, 20 bp, synthetic construct
  misc_feature 1..20: note = Primer for DELTAgene qPCR assay in Example 2
  source 1..20: mol_type = other DNA
gagcagggttctgggcttta

SEQ ID NO: 35 - DNA, 20 bp, synthetic construct
  misc_feature 1..20: note = Primer for DELTAgene qPCR assay in Example 2
  source 1..20: mol_type = other DNA
cactactgggctcagggaaa

SEQ ID NO: 36 - DNA, 19 bp, synthetic construct
  misc_feature 1..19: note = Primer for DELTAgene qPCR assay in Example 2
  source 1..19: mol_type = other DNA
tgctggtcacagtccttca

SEQ ID NO: 37 - DNA, 20 bp, synthetic construct
  misc_feature 1..20: note = Primer for DELTAgene qPCR assay in Example 2
  source 1..20: mol_type = other DNA
gtcctggcttgctatagctt

SEQ ID NO: 38 - DNA, 20 bp, synthetic construct
  misc_feature 1..20: note = Primer for DELTAgene qPCR assay in Example 2
  source 1..20: mol_type = other DNA
catgtagtcactgtgcagga

SEQ ID NO: 39 - DNA, 19 bp, synthetic construct
  misc_feature 1..19: note = Primer for DELTAgene qPCR assay in Example 2
  source 1..19: mol_type = other DNA
cgtttctctctggcctggt

SEQ ID NO: 40 - DNA, 22 bp, synthetic construct
  misc_feature 1..22: note = Primer for DELTAgene qPCR assay in Example 2
  source 1..22: mol_type = other DNA
ctctacccatgtgatgctggta

SEQ ID NO: 41 - DNA, 20 bp, synthetic construct
  misc_feature 1..20: note = Primer for DELTAgene qPCR assay in Example 2
  source 1..20: mol_type = other DNA
gctaccccagaggaagcaaa

SEQ ID NO: 42 - DNA, 22 bp, synthetic construct
  misc_feature 1..22: note = Primer for DELTAgene qPCR assay in Example 2
  source 1..22: mol_type = other DNA
tccatctccatgcagttctcac

SEQ ID NO: 43 - DNA, 23 bp, synthetic construct
  misc_feature 1..23: note = Primer for DELTAgene qPCR assay in Example 2
  source 1..23: mol_type = other DNA
aaagttgcatcaggaagtgaacc

SEQ ID NO: 44 - DNA, 20 bp, synthetic construct
  misc_feature 1..20: note = Primer for DELTAgene qPCR assay in Example 2
  source 1..20: mol_type = other DNA
cccacacctcacaggtcaaa

SEQ ID NO: 45 - DNA, 20 bp, synthetic construct
  misc_feature 1..20: note = Primer for DELTAgene qPCR assay in Example 2
  source 1..20: mol_type = other DNA
gaggccagcagtaaaacaac

SEQ ID NO: 46 - DNA, 22 bp, synthetic construct
  misc_feature 1..22: note = Primer for DELTAgene qPCR assay in Example 2
  source 1..22: mol_type = other DNA
agttgttgctcatggtgtagta

SEQ ID NO: 47 - DNA, 20 bp, synthetic construct
  misc_feature 1..20: note = Primer for DELTAgene qPCR assay in Example 2
  source 1..20: mol_type = other DNA
ccggacaccatggacaagtt

SEQ ID NO: 48 - DNA, 17 bp, synthetic construct
  misc_feature 1..17: note = Primer for DELTAgene qPCR assay in Example 2
  source 1..17: mol_type = other DNA
cctgcaaagcggcaggt

SEQ ID NO: 49 - DNA, 24 bp, synthetic construct
  misc_feature 1..24: note = Primer for DELTAgene qPCR assay in Example 2
  source 1..24: mol_type = other DNA
aatcattttgacaacctgtatccc

SEQ ID NO: 50 - DNA, 26 bp, synthetic construct
  misc_feature 1..26: note = Primer for DELTAgene qPCR assay in Example 2
  source 1..26: mol_type = other DNA
tgtaattactgctaatggtatgggta

SEQ ID NO: 51 - DNA, 17 bp, synthetic construct
  misc_feature 1..17: note = Primer for DELTAgene qPCR assay in Example 2
  source 1..17: mol_type = other DNA
gcagccagccttgggaa

SEQ ID NO: 52 - DNA, 25 bp, synthetic construct
  misc_feature 1..25: note = Primer for DELTAgene qPCR assay in Example 2
  source 1..25: mol_type = other DNA
gcaagaacttcacacatttcattcc

SEQ ID NO: 53 - DNA, 20 bp, synthetic construct
  misc_feature 1..20: note = Primer for DELTAgene qPCR assay in Example 2
  source 1..20: mol_type = other DNA
tcacccatggaagtggtcaa

SEQ ID NO: 54 - DNA, 21 bp, synthetic construct
  misc_feature 1..21: note = Primer for DELTAgene qPCR assay in Example 2
  source 1..21: mol_type = other DNA
acacacttgtcagaccctgta

SEQ ID NO: 55 - DNA, 19 bp, synthetic construct
  misc_feature 1..19: note = Primer for DELTAgene qPCR assay in Example 2
  source 1..19: mol_type = other DNA
tgctggctggtctttctca

SEQ ID NO: 56 - DNA, 21 bp, synthetic construct
  misc_feature 1..21: note = Primer for DELTAgene qPCR assay in Example 2
  source 1..21: mol_type = other DNA
gagtttgtgccagctcttcaa

SEQ ID NO: 57 - DNA, 19 bp, synthetic construct
  misc_feature 1..19: note = Primer for DELTAgene qPCR assay in Example 2
  source 1..19: mol_type = other DNA
cggcctcgcaactcttata

SEQ ID NO: 58 - DNA, 20 bp, synthetic construct
  misc_feature 1..20: note = Primer for DELTAgene qPCR assay in Example 2
  source 1..20: mol_type = other DNA
tggtctgttcactctcttcc

SEQ ID NO: 59 - DNA, 19 bp, synthetic construct
  misc_feature 1..19: note = Primer for DELTAgene qPCR assay in Example 2
  source 1..19: mol_type = other DNA
acttcgtgccggtcttcct

SEQ ID NO: 60 - DNA, 16 bp, synthetic construct
  misc_feature 1..16: note = Primer for DELTAgene qPCR assay in Example 2
  source 1..16: mol_type = other DNA
gctgcgacgcgatggt

SEQ ID NO: 61 - DNA, 19 bp, synthetic construct
  misc_feature 1..19: note = Primer for DELTAgene qPCR assay in Example 2
  source 1..19: mol_type = other DNA
tgatggccagccactacaa

SEQ ID NO: 62 - DNA, 22 bp, synthetic construct
  misc_feature 1..22: note = Primer for DELTAgene qPCR assay in Example 2
  source 1..22: mol_type = other DNA
caaaggggatgacaagcagaaa

SEQ ID NO: 63 - DNA, 20 bp, synthetic construct
  misc_feature 1..20: note = Primer for DELTAgene qPCR assay in Example 2
  source 1..20: mol_type = other DNA
cttggatttcagcggcacaa

SEQ ID NO: 64 - DNA, 17 bp, synthetic construct
  misc_feature 1..17: note = Primer for DELTAgene qPCR assay in Example 2
  source 1..17: mol_type = other DNA
gctgctggccagtacca

SEQ ID NO: 65 - DNA, 19 bp, synthetic construct
  misc_feature 1..19: note = Primer for DELTAgene qPCR assay in Example 2
  source 1..19: mol_type = other DNA
ccaccttctgccatctgac

SEQ ID NO: 66 - DNA, 21 bp, synthetic construct
  misc_feature 1..21: note = Primer for DELTAgene qPCR assay in Example 2
  source 1..21: mol_type = other DNA
cgtgatgttgcatttcgtcac

SEQ ID NO: 67 - DNA, 21 bp, synthetic construct
  misc_feature 1..21: note = Primer for DELTAgene qPCR assay in Example 2
  source 1..21: mol_type = other DNA
gtagtgtttgccctcaccaac

SEQ ID NO: 68 - DNA, 20 bp, synthetic construct
  misc_feature 1..20: note = Primer for DELTAgene qPCR assay in Example 2
  source 1..20: mol_type = other DNA
atcagacaaggccaggttca

SEQ ID NO: 69 - DNA, 21 bp, synthetic construct
  misc_feature 1..21: note = Primer for DELTAgene qPCR assay in Example 2
  source 1..21: mol_type = other DNA
gctgtacctgcatcagcatta

SEQ ID NO: 70 - DNA, 23 bp, synthetic construct
  misc_feature 1..23: note = Primer for DELTAgene qPCR assay in Example 2
  source 1..23: mol_type = other DNA
ctggattcagacatctcttctac

SEQ ID NO: 71 - DNA, 20 bp, synthetic construct
  misc_feature 1..20: note = Primer for DELTAgene qPCR assay in Example 2
  source 1..20: mol_type = other DNA
agccaacgtcaagcatctca

SEQ ID NO: 72 - DNA, 19 bp, synthetic construct
  misc_feature 1..19: note = Primer for DELTAgene qPCR assay in Example 2
  source 1..19: mol_type = other DNA
gcttcgggtcaatgcacac

SEQ ID NO: 73 - DNA, 19 bp, synthetic construct
  misc_feature 1..19: note = Primer for DELTAgene qPCR assay in Example 2
  source 1..19: mol_type = other DNA
agcccttcctgcgagaaaa

SEQ ID NO: 74 - DNA, 24 bp, synthetic construct
  misc_feature 1..24: note = Primer for DELTAgene qPCR assay in Example 2
  source 1..24: mol_type = other DNA
atctgctgaatctgggtttagaca

SEQ ID NO: 75 - DNA, 20 bp, synthetic construct
  misc_feature 1..20: note = Primer for DELTAgene qPCR assay in Example 2
  source 1..20: mol_type = other DNA
atctctgactgcagctccta

SEQ ID NO: 76 - DNA, 21 bp, synthetic construct
  misc_feature 1..21: note = Primer for DELTAgene qPCR assay in Example 2
  source 1..21: mol_type = other DNA
tgtcctcttcagtttcagcaa

SEQ ID NO: 77 - DNA, 19 bp, synthetic construct
  misc_feature 1..19: note = Primer for DELTAgene qPCR assay in Example 2
  source 1..19: mol_type = other DNA
aactgtggccgagaaagca

SEQ ID NO: 78 - DNA, 20 bp, synthetic construct
  misc_feature 1..20: note = Primer for DELTAgene qPCR assay in Example 2
  source 1..20: mol_type = other DNA
ttgaggcagcagtgcatgta

SEQ ID NO: 79 - DNA, 21 bp, synthetic construct
  misc_feature 1..21: note = Primer for DELTAgene qPCR assay in Example 2
  source 1..21: mol_type = other DNA
atcttcctgcccaccatctac

SEQ ID NO: 80 - DNA, 20 bp, synthetic construct
  misc_feature 1..20: note = Primer for DELTAgene qPCR assay in Example 2
  source 1..20: mol_type = other DNA
cccatgaccaggatgaccaa

SEQ ID NO: 81 - DNA, 21 bp, synthetic construct
  misc_feature 1..21: note = Primer for DELTAgene qPCR assay in Example 2
  source 1..21: mol_type = other DNA
tggggatgtttcagctcttcc

SEQ ID NO: 82 - DNA, 20 bp, synthetic construct
  misc_feature 1..20: note = Primer for DELTAgene qPCR assay in Example 2
  source 1..20: mol_type = other DNA
ctgtgtgcatctggctggta

SEQ ID NO: 83 - DNA, 19 bp, synthetic construct
  misc_feature 1..19: note = Primer for DELTAgene qPCR assay in Example 2
  source 1..19: mol_type = other DNA
tgtggggtagccatggaaa

SEQ ID NO: 84 - DNA, 18 bp, synthetic construct
  misc_feature 1..18: note = Primer for DELTAgene qPCR assay in Example 2
  source 1..18: mol_type = other DNA
gggtcgcatgttgtggaa

SEQ ID NO: 85 - DNA, 20 bp, synthetic construct
  misc_feature 1..20: note = Primer for DELTAgene qPCR assay in Example 2
  source 1..20: mol_type = other DNA
gccgtcaccaagaacattca

SEQ ID NO: 86 - DNA, 18 bp, synthetic construct
  misc_feature 1..18: note = Primer for DELTAgene qPCR assay in Example 2
  source 1..18: mol_type = other DNA
ctcccgaagggcttctcc

SEQ ID NO: 87 - DNA, 20 bp, synthetic construct
  misc_feature 1..20: note = Primer for DELTAgene qPCR assay in Example 2
  source 1..20: mol_type = other DNA
acaccatggggaaggtgaag

SEQ ID NO: 88 - DNA, 18 bp, synthetic construct
  misc_feature 1..18: note = Primer for DELTAgene qPCR assay in Example 2
  source 1..18: mol_type = other DNA
gtgaccaggcgcccaata

SEQ ID NO: 89 - DNA, 18 bp, synthetic construct
  misc_feature 1..18: note = Primer for DELTAgene qPCR assay in Example 2
  source 1..18: mol_type = other DNA
cacggtgcagaggtaccc

SEQ ID NO: 90 - DNA, 21 bp, synthetic construct
  misc_feature 1..21: note = Primer for DELTAgene qPCR assay in Example 2
  source 1..21: mol_type = other DNA
agggtagggatccatgaagca

SEQ ID NO: 91 - DNA, 18 bp, synthetic construct
  misc_feature 1..18: note = Primer for DELTAgene qPCR assay in Example 2
  source 1..18: mol_type = other DNA
gaagcctccgaggtggaa

SEQ ID NO: 92 - DNA, 20 bp, synthetic construct
  misc_feature 1..20: note = Primer for DELTAgene qPCR assay in Example 2
  source 1..20: mol_type = other DNA
gaaaacaccctcgcacaaca

SEQ ID NO: 93 - DNA, 23 bp, synthetic construct
  misc_feature 1..23: note = Primer for DELTAgene qPCR assay in Example 2
  source 1..23: mol_type = other DNA
ccccatccagcctataatcctaa

SEQ ID NO: 94 - DNA, 20 bp, synthetic construct
  misc_feature 1..20: note = Primer for DELTAgene qPCR assay in Example 2
  source 1..20: mol_type = other DNA
ctgggccttgttgctaggta

SEQ ID NO: 95 - DNA, 19 bp, synthetic construct
  misc_feature 1..19: note = Primer for DELTAgene qPCR assay in Example 2
  source 1..19: mol_type = other DNA
atccacagtgggtgctgac

SEQ ID NO: 96 - DNA, 20 bp, synthetic construct
  misc_feature 1..20: note = Primer for DELTAgene qPCR assay in Example 2
  source 1..20: mol_type = other DNA
agagtgtgcgcctaaaacca

SEQ ID NO: 97 - DNA, 21 bp, synthetic construct
  misc_feature 1..21: note = Primer for DELTAgene qPCR assay in Example 2
  source 1..21: mol_type = other DNA
ggatccaaatcccaggcataa

SEQ ID NO: 98 - DNA, 20 bp, synthetic construct
  misc_feature 1..20: note = Primer for DELTAgene qPCR assay in Example 2
  source 1..20: mol_type = other DNA
cttggaaaggctgcagtgaa

SEQ ID NO: 99 - DNA, 20 bp, synthetic construct
  misc_feature 1..20: note = Primer for DELTAgene qPCR assay in Example 2
  source 1..20: mol_type = other DNA
agtctgcattttgggatgca

SEQ ID NO: 100 - DNA, 19 bp, synthetic construct
  misc_feature 1..19: note = Primer for DELTAgene qPCR assay in Example 2
  source 1..19: mol_type = other DNA
gtcgtgcacactggatgaa

SEQ ID NO: 101 - DNA, 20 bp, synthetic construct
  misc_feature 1..20: note = Primer for DELTAgene qPCR assay in Example 2
  source 1..20: mol_type = other DNA
ttggctgctgcatagagaac

SEQ ID NO: 102 - DNA, 22 bp, synthetic construct
  misc_feature 1..22: note = Primer for DELTAgene qPCR assay in Example 2
  source 1..22: mol_type = other DNA
cttgtctctctctccgatgtca

SEQ ID NO: 103 - DNA, 21 bp, synthetic construct
  misc_feature 1..21: note = Primer for DELTAgene qPCR assay in Example 2
  source 1..21: mol_type = other DNA
actgccaggacccatatgtaa

SEQ ID NO: 104 - DNA, 26 bp, synthetic construct
  misc_feature 1..26: note = Primer for DELTAgene qPCR assay in Example 2
  source 1..26: mol_type = other DNA
gttccattatatccgctacatctgaa

SEQ ID NO: 105 - DNA, 19 bp, synthetic construct
  misc_feature 1..19: note = Primer for DELTAgene qPCR assay in Example 2
  source 1..19: mol_type = other DNA
aagttagggttggacaaaa

SEQ ID NO: 106 - DNA, 23 bp, synthetic construct
  misc_feature 1..23: note = Primer for DELTAgene qPCR assay in Example 2
  source 1..23: mol_type = other DNA
gatatccagtttaggtggtccaa

SEQ ID NO: 107 - DNA, 19 bp, synthetic construct
  misc_feature 1..19: note = Primer for DELTAgene qPCR assay in Example 2
  source 1..19: mol_type = other DNA
ccgtggagcaggtgaagaa

SEQ ID NO: 108 - DNA, 24 bp, synthetic construct
  misc_feature 1..24: note = Primer for DELTAgene qPCR assay in Example 2
  source 1..24: mol_type = other DNA
gtcaaactcactcatggctttgta

SEQ ID NO: 109 - DNA, 19 bp, synthetic construct
  misc_feature 1..19: note = Primer for DELTAgene qPCR assay in Example 2
  source 1..19: mol_type = other DNA
cacagtggaggcctgttta

SEQ ID NO: 110 - DNA, 22 bp, synthetic construct
  misc_feature 1..22: note = Primer for DELTAgene qPCR assay in Example 2
  source 1..22: mol_type = other DNA
tctggaatttaggcaactctca

SEQ ID NO: 111 - DNA, 20 bp, synthetic construct
  misc_feature 1..20: note = Primer for DELTAgene qPCR assay in Example 2
  source 1..20: mol_type = other DNA
tccctgacattctgcgttca

SEQ ID NO: 112 - DNA, 22 bp, synthetic construct
  misc_feature 1..22: note = Primer for DELTAgene qPCR assay in Example 2
  source 1..22: mol_type = other DNA
ggtcttgtccgtgaagactcta

SEQ ID NO: 113 - DNA, 19 bp, synthetic construct
  misc_feature 1..19: note = Primer for DELTAgene qPCR assay in Example 2
  source 1..19: mol_type = other DNA
gccatatccggatgcagac

SEQ ID NO: 114 - DNA, 19 bp, synthetic construct
  misc_feature 1..19: note = Primer for DELTAgene qPCR assay in Example 2
  source 1..19: mol_type = other DNA
cagctgtgggaccctcata

SEQ ID NO: 115 - DNA, 21 bp, synthetic construct
  misc_feature 1..21: note = Primer for DELTAgene qPCR assay in Example 2
  source 1..21: mol_type = other DNA
gtcttggaagctcctcttcac

SEQ ID NO: 116 - DNA, 20 bp, synthetic construct
  misc_feature 1..20: note = Primer for DELTAgene qPCR assay in Example 2
  source 1..20: mol_type = other DNA
tctaatgtcccacggaggaa

SEQ ID NO: 117 - DNA, 20 bp, synthetic construct
  misc_feature 1..20: note = Primer for DELTAgene qPCR assay in Example 2
  source 1..20: mol_type = other DNA
tgcagtgccatcgagaagac

SEQ ID NO: 118 - DNA, 20 bp, synthetic construct
  misc_feature 1..20: note = Primer for DELTAgene qPCR assay in Example 2
  source 1..20: mol_type = other DNA
tcggacatgcaagctggaaa

SEQ ID NO: 119 - DNA, 20 bp, synthetic construct
  misc_feature 1..20: note = Primer for DELTAgene qPCR assay in Example 2
  source 1..20: mol_type = other DNA
agccaactgggtgaatgtaa

SEQ ID NO: 120 - DNA, 26 bp, synthetic construct
  misc_feature 1..26: note = Primer for DELTAgene qPCR assay in Example 2
  source 1..26: mol_type = other DNA
cactttccgtatataaagtagcatca

SEQ ID NO: 121 - DNA, 18 bp, synthetic construct
  misc_feature 1..18: note = Primer for DELTAgene qPCR assay in Example 2
  source 1..18: mol_type = other DNA
tgagcgctgtgtctctcc

SEQ ID NO: 122 - DNA, 22 bp, synthetic construct
  misc_feature 1..22: note = Primer for DELTAgene qPCR assay in Example 2
  source 1..22: mol_type = other DNA
cctccatggcttccatttcaac

SEQ ID NO: 123 - DNA, 21 bp, synthetic construct
  misc_feature 1..21: note = Primer for DELTAgene qPCR assay in Example 2
  source 1..21: mol_type = other DNA
actacaaccgatccacctcac

SEQ ID NO: 124 - DNA, 20 bp, synthetic construct
  misc_feature 1..20: note = Primer for DELTAgene qPCR assay in Example 2
  source 1..20: mol_type = other DNA
actttgcctcccagatcaca

SEQ ID NO: 125 - DNA, 20 bp, synthetic construct
  misc_feature 1..20: note = Primer for DELTAgene qPCR assay in Example 2
  source 1..20: mol_type = other DNA
ctgtggcaaagccgacaata

SEQ ID NO: 126 - DNA, 21 bp, synthetic construct
  misc_feature 1..21: note = Primer for DELTAgene qPCR assay in Example 2
  source 1..21: mol_type = other DNA
ctcatccagtgggaaccagta

SEQ ID NO: 127 - DNA, 20 bp, synthetic construct
  misc_feature 1..20: note = Primer for DELTAgene qPCR assay in Example 2
  source 1..20: mol_type = other DNA
ccaaaccaccagtccaagaa

SEQ ID NO: 128 - DNA, 19 bp, synthetic construct
  misc_feature 1..19: note = Primer for DELTAgene qPCR assay in Example 2
  source 1..19: mol_type = other DNA
ctcatgcatggcgtggtta

SEQ ID NO: 129 - DNA, 21 bp, synthetic construct
  misc_feature 1..21: note = Primer for DELTAgene qPCR assay in Example 2
  source 1..21: mol_type = other DNA
gaccaaggaaatcggcctcta

SEQ ID NO: 130 - DNA, 25 bp, synthetic construct
  misc_feature 1..25: note = Primer for DELTAgene qPCR assay in Example 2
  source 1..25: mol_type = other DNA
tcacagagatagttacagccatacc

SEQ ID NO: 131 - DNA, 24 bp, synthetic construct
  misc_feature 1..24: note = Primer for DELTAgene qPCR assay in Example 2
  source 1..24: mol_type = other DNA
cgttcttcttggaccaaagcttaa

SEQ ID NO: 132 - DNA, 20 bp, synthetic construct
  misc_feature 1..20: note = Primer for DELTAgene qPCR assay in Example 2
  source 1..20: mol_type = other DNA
agcagagcagttgagcctta

SEQ ID NO: 133 - DNA, 22 bp, synthetic construct
  misc_feature 1..22: note = Primer for DELTAgene qPCR assay in Example 2
  source 1..22: mol_type = other DNA
cccagggacttaatcagcaata

SEQ ID NO: 134 - DNA, 22 bp, synthetic construct
  misc_feature 1..22: note = Primer for DELTAgene qPCR assay in Example 2
  source 1..22: mol_type = other DNA
ttctacaatggttgctgtctca

SEQ ID NO: 135 - DNA, 21 bp, synthetic construct
  misc_feature 1..21: note = Primer for DELTAgene qPCR assay in Example 2
  source 1..21: mol_type = other DNA
tgcatcctggaaatgtggaac

SEQ ID NO: 136 - DNA, 22 bp, synthetic construct
  misc_feature 1..22: note = Primer for DELTAgene qPCR assay in Example 2
  source 1..22: mol_type = other DNA
cctcgtccttcagctcttcata

SEQ ID NO: 137 - DNA, 20 bp, synthetic construct
  misc_feature 1..20: note = Primer for DELTAgene qPCR assay in Example 2
  source 1..20: mol_type = other DNA
gcacaggtgaaatggagacc

SEQ ID NO: 138 - DNA, 19 bp, synthetic construct
  misc_feature 1..19: note = Primer for DELTAgene qPCR assay in Example 2
  source 1..19: mol_type = other DNA
gacgaggcaggaagtctca

SEQ ID NO: 139 - DNA, 20 bp, synthetic construct
  misc_feature 1..20: note = Primer for DELTAgene qPCR assay in Example 2
  source 1..20: mol_type = other DNA
atggccatccaggacttaca

SEQ ID NO: 140 - DNA, 19 bp, synthetic construct
  misc_feature 1..19: note = Primer for DELTAgene qPCR assay in Example 2
  source 1..19: mol_type = other DNA
ttgcatctgtgggtctcca

SEQ ID NO: 141 - DNA, 20 bp, synthetic construct
  misc_feature 1..20: note = Primer for DELTAgene qPCR assay in Example 2
  source 1..20: mol_type = other DNA
gcccaatgggaatgaagaca

SEQ ID NO: 142 - DNA, 20 bp, synthetic construct
  misc_feature 1..20: note = Primer for DELTAgene qPCR assay in Example 2
  source 1..20: mol_type = other DNA
tggaaacactgagggagtca

SEQ ID NO: 143 - DNA, 21 bp, synthetic construct
  misc_feature 1..21: note = Primer for DELTAgene qPCR assay in Example 2
  source 1..21: mol_type = other DNA
cagctgatccgattcctgaaa

SEQ ID NO: 144 - DNA, 20 bp, synthetic construct
  misc_feature 1..20: note = Primer for DELTAgene qPCR assay in Example 2
  source 1..20: mol_type = other DNA
gttggcttccttcacaggac

SEQ ID NO: 145 - DNA, 19 bp, synthetic construct
  misc_feature 1..19: note = Primer for DELTAgene qPCR assay in Example 2
  source 1..19: mol_type = other DNA
gagctccgcctgttgtacc

SEQ ID NO: 146 - DNA, 18 bp, synthetic construct
  misc_feature 1..18: note = Primer for DELTAgene qPCR assay in Example 2
  source 1..18: mol_type = other DNA
gcgcctccgttgttctca

SEQ ID NO: 147 - DNA, 24 bp, synthetic construct
  misc_feature 1..24: note = Primer for DELTAgene qPCR assay in Example 2
  source 1..24: mol_type = other DNA
actctgaggattcctgttcctgta

SEQ ID NO: 148 - DNA, 22 bp, synthetic construct
  misc_feature 1..22: note = Primer for DELTAgene qPCR assay in Example 2
  source 1..22: mol_type = other DNA
ccagtgtgcctattccctgaaa

SEQ ID NO: 149 - DNA, 21 bp, synthetic construct
  misc_feature 1..21: note = Primer for DELTAgene qPCR assay in Example 2
  source 1..21: mol_type = other DNA
ggagaaagtggctatgctcaa

SEQ ID NO: 150 - DNA, 20 bp, synthetic construct
  misc_feature 1..20: note = Primer for DELTAgene qPCR assay in Example 2
  source 1..20: mol_type = other DNA
ctgcgatccattcacttcca

SEQ ID NO: 151 - DNA, 19 bp, synthetic construct
  misc_feature 1..19: note = Primer for DELTAgene qPCR assay in Example 2
  source 1..19: mol_type = other DNA
ctacaaccgcgaggaggac

SEQ ID NO: 152 - DNA, 20 bp, synthetic construct
  misc_feature 1..20: note = Primer for DELTAgene qPCR assay in Example 2
  source 1..20: mol_type = other DNA
tgtcgatgccttctcggaac

SEQ ID NO: 153 - DNA, 20 bp, synthetic construct
  misc_feature 1..20: note = Primer for DELTAgene qPCR assay in Example 2
  source 1..20: mol_type = other DNA
ctgcggcaaaacctacacaa

SEQ ID NO: 154 - DNA, 20 bp, synthetic construct
  misc_feature 1..20: note = Primer for DELTAgene qPCR assay in Example 2
  source 1..20: mol_type = other DNA
cgtcccagtcacagtggtaa

SEQ ID NO: 155 - DNA, 20 bp, synthetic construct
  misc_feature 1..20: note = Primer for DELTAgene qPCR assay in Example 2
  source 1..20: mol_type = other DNA
acccaagcccagaatgacta

SEQ ID NO: 156 - DNA, 19 bp, synthetic construct
  misc_feature 1..19: note = Primer for DELTAgene qPCR assay in Example 2
  source 1..19: mol_type = other DNA
ttgccacaaggcaagaaca

SEQ ID NO: 157 - DNA, 19 bp, synthetic construct
  misc_feature 1..19: note = Primer for DELTAgene qPCR assay in Example 2
  source 1..19: mol_type = other DNA
tggagcctttggctttcac

SEQ ID NO: 158 - DNA, 21 bp, synthetic construct
  misc_feature 1..21: note = Primer for DELTAgene qPCR assay in Example 2
  source 1..21: mol_type = other DNA
gagggtgaatcccttgctcta

SEQ ID NO: 159 - DNA, 22 bp, synthetic construct
  misc_feature 1..22: note = Primer for DELTAgene qPCR assay in Example 2
  source 1..22: mol_type = other DNA
aagaaagtgcagctatcaacca

SEQ ID NO: 160 - DNA, 21 bp, synthetic construct
  misc_feature 1..21: note = Primer for DELTAgene qPCR assay in Example 2
  source 1..21: mol_type = other DNA
gctgtctttctttccgtgcta

SEQ ID NO: 161 - DNA, 20 bp, synthetic construct
  misc_feature 1..20: note = Primer for DELTAgene qPCR assay in Example 2
  source 1..20: mol_type = other DNA
tgtcccatcctgaggcacta

SEQ ID NO: 162 - DNA, 19 bp, synthetic construct
  misc_feature 1..19: note = Primer for DELTAgene qPCR assay in Example 2
  source 1..19: mol_type = other DNA
accgttaagcgggcagtac

SEQ ID NO: 163 - DNA, 21 bp, synthetic construct
  misc_feature 1..21: note = Primer for DELTAgene qPCR assay in Example 2
  source 1..21: mol_type = other DNA
ctggaaccacgcctctagata

SEQ ID NO: 164 - DNA, 23 bp, synthetic construct
  misc_feature 1..23: note = Primer for DELTAgene qPCR assay in Example 2
  source 1..23: mol_type = other DNA
aaactctggctcatatggtttcc

SEQ ID NO: 165 - DNA, 17 bp, synthetic construct
  misc_feature 1..17: note = Primer for DELTAgene qPCR assay in Example 2
  source 1..17: mol_type = other DNA
gcagcctggtgctgcta

SEQ ID NO: 166 - DNA, 16 bp, synthetic construct
  misc_feature 1..16: note = Primer for DELTAgene qPCR assay in Example 2
  source 1..16: mol_type = other DNA
gtgcgcctggctccta

SEQ ID NO: 167 - DNA, 21 bp, synthetic construct
  misc_feature 1..21: note = Primer for DELTAgene qPCR assay in Example 2
  source 1..21: mol_type = other DNA
gtacagcttcagcactgacac

SEQ ID NO: 168 - DNA, 18 bp, synthetic construct
  misc_feature 1..18: note = Primer for DELTAgene qPCR assay in Example 2
  source 1..18: mol_type = other DNA
ctgggtggaggcgttgaa

SEQ ID NO: 169 - DNA, 20 bp, synthetic construct
  misc_feature 1..20: note = Primer for DELTAgene qPCR assay in Example 2
  source 1..20: mol_type = other DNA
cagcagataacgtggcagac

SEQ ID NO: 170 - DNA, 20 bp, synthetic construct
  misc_feature 1..20: note = Primer for DELTAgene qPCR assay in Example 2
  source 1..20: mol_type = other DNA
ggcacacaattgccacatca

SEQ ID NO: 171 - DNA, 19 bp, synthetic construct
  misc_feature 1..19: note = Primer for DELTAgene qPCR assay in Example 2
  source 1..19: mol_type = other DNA
cagactcatcgccaaagca

SEQ ID NO: 172 - DNA, 20 bp, synthetic construct
  misc_feature 1..20: note = Primer for DELTAgene qPCR assay in Example 2
  source 1..20: mol_type = other DNA
tttccacatgctggctacac

SEQ ID NO: 173 - DNA, 22 bp, synthetic construct
  misc_feature 1..22: note = Primer for DELTAgene qPCR assay in Example 2
  source 1..22: mol_type = other DNA
cccaggctccctataacatgta

SEQ ID NO: 174 - DNA, 20 bp, synthetic construct
  misc_feature 1..20: note = Primer for DELTAgene qPCR assay in Example 2
  source 1..20: mol_type = other DNA
atggtctcatccaggtcgaa

SEQ ID NO: 175 - DNA, 20 bp, synthetic construct
  misc_feature 1..20: note = Primer for DELTAgene qPCR assay in Example 2
  source 1..20: mol_type = other DNA
aacagaggttggtccgagaa

SEQ ID NO: 176 - DNA, 20 bp, synthetic construct
  misc_feature 1..20: note = Primer for DELTAgene qPCR assay in Example 2
  source 1..20: mol_type = other DNA
gtttctgggacatggcatca

SEQ ID NO: 177 - DNA, 23 bp, synthetic construct
  misc_feature 1..23: note = Primer for DELTAgene qPCR assay in Example 2
  source 1..23: mol_type = other DNA
ttcaatctgctcatgcattaccc

SEQ ID NO: 178 - DNA, 22 bp, synthetic construct
  misc_feature 1..22: note = Primer for DELTAgene qPCR assay in Example 2
  source 1..22: mol_type = other DNA
gtgggctgttgaaatgttcgta

SEQ ID NO: 179 - DNA, 21 bp, synthetic construct
  misc_feature 1..21: note = Primer for DELTAgene qPCR assay in Example 2
  source 1..21: mol_type = other DNA
cgtctgctgaggctcaagtta

SEQ ID NO: 180 - DNA, 21 bp, synthetic construct
  misc_feature 1..21: note = Primer for DELTAgene qPCR assay in Example 2
  source 1..21: mol_type = other DNA
tcgccaggaattgttgctgta

SEQ ID NO: 181 - DNA, 20 bp, synthetic construct
  misc_feature 1..20: note = Primer for DELTAgene qPCR assay in Example 2
  source 1..20: mol_type = other DNA
caaaagccagagtgcctgaa

SEQ ID NO: 182 - DNA, 21 bp, synthetic construct
  misc_feature 1..21: note = Primer for DELTAgene qPCR assay in Example 2
  source 1..21: mol_type = other DNA
cgctgggttggagatgttaaa

SEQ ID NO: 183 - DNA, 21 bp, synthetic construct
  misc_feature 1..21: note = Primer for DELTAgene qPCR assay in Example 2
  source 1..21: mol_type = other DNA
gaaattgctcgacgatgttcc

SEQ ID NO: 184 - DNA, 21 bp, synthetic construct
  misc_feature 1..21: note = Primer for DELTAgene qPCR assay in Example 2
  source 1..21: mol_type = other DNA
actgatgggtcagaaggtaca

SEQ ID NO: 185 - DNA, 22 bp, synthetic construct
  misc_feature 1..22: note = Primer for DELTAgene qPCR assay in Example 2
  source 1..22: mol_type = other DNA
ggggcagaaagaaactcctgta

SEQ ID NO: 186 - DNA, 20 bp, synthetic construct
  misc_feature 1..20: note = Primer for DELTAgene qPCR assay in Example 2
  source 1..20: mol_type = other DNA
tctggaaatcggcagctaca

SEQ ID NO: 187 - DNA, 19 bp, synthetic construct
  misc_feature 1..19: note = Primer for DELTAgene qPCR assay in Example 2
  source 1..19: mol_type = other DNA
aggtctcacgaggtcaacc

SEQ ID NO: 188 - DNA, 20 bp, synthetic construct
  misc_feature 1..20: note = Primer for DELTAgene qPCR assay in Example 2
  source 1..20: mol_type = other DNA
cccagctgagtctcccataa

SEQ ID NO: 189 - DNA, 21 bp, synthetic construct
  misc_feature 1..21: note = Primer for DELTAgene qPCR assay in Example 2
  source 1..21: mol_type = other DNA
aagcgcgataacctcctcata

SEQ ID NO: 190 - DNA, 19 bp, synthetic construct
  misc_feature 1..19: note = Primer for DELTAgene qPCR assay in Example 2
  source 1..19: mol_type = other DNA
ttccgtgtctgccttctcc